European Patent Application EP 4 509 129 A1, published February 19, 2025. Title: GLUCURONIDASE ACTIVATOR, PHARMACEUTICAL COMPOSITION, DIETARY COMPOSITION AND COMPOSITION FOR ORAL USE. Applicant: 株式会社カネカ. Application JP. The sequence listing filed with the application follows.

SEQUENCE LISTING (6 sequences)

SEQ ID NO: 1 - DNA, 19 bp, synthetic construct
  misc_feature 1..19: note = forward Eub27f primer
  source 1..19: mol_type = other DNA
gagtttgatcctggctcag

SEQ ID NO: 2 - DNA, 22 bp, synthetic construct
  misc_feature 1..22: note = reverse Eub1492r primer
  source 1..22: mol_type = other DNA
tacggytaccttgttacgactt

SEQ ID NO: 3 - DNA, 20 bp, synthetic construct
  misc_feature 1..20: note = forward 27f primer
  source 1..20: mol_type = other DNA
agagtttgatcctggctcag

SEQ ID NO: 4 - DNA, 57 bp, synthetic construct
  misc_feature 1..57: note = forward 357f primer
  source 1..57: mol_type = other DNA
cgcccgccgcgccccgcgcccggcccgccgcccccgcccccctacgggaggcagcag

SEQ ID NO: 5 - DNA, 20 bp, synthetic construct
  misc_feature 1..20: note = reverse 907r primer
  source 1..20: mol_type = other DNA
ccgtcaattcctttgagttt

SEQ ID NO: 6 - DNA, 19 bp, synthetic construct
  misc_feature 1..19: note = reverse 1492r primer
  source 1..19: mol_type = other DNA
ggttaccttgttacgactt